European Patent Application EP 4 613 291 A1, published September 10, 2025. Title: 항-클라우딘18.2 항체를 포함하는 항체-약물 컨쥬게이트 및 이의 암에 대한 치료용도. Applicant: 앱티스 주식회사. The sequence listing filed with the application follows.

SEQUENCE LISTING (19 sequences)

SEQ ID NO: 1 - protein, 208 aa, synthetic construct
  source 1..208: note = Fc region of Claudin18.2 antibody
GPSVFLFPPKPKDTLMISRTPEVTCVVVDVSHEDPEVKFNWYVDGVEVHNAKTKPREEQYNSTYRVVSVLTVLHQDWLNGKEYKCKVSNKALPAPIEKTISKAKGQPREPQVYTLPPSRDELTKNQVSLTCLVKGFYPSDIAVEWESNGQPENNYKTTPPVLDSDGSFFLYSKLTVDKSRWQQGNVFSCSVMHEALHNHYTQKSLSLS

SEQ ID NO: 2 - protein, 208 aa, synthetic construct
  source 1..208: note = Fc region of IgG1
GPSVFLFPPKPKDTLMISRTPEVTCVVVDVSHEDPEVKFNWYVDGVEVHNAKTKPREEQYNSTYRVVSVLTVLHQDWLNGKEYKCKVSNKALPAPIEKTISKAKGQPREPQVYTLPPSREEMTKNQVSLTCLVKGFYPSDIAVEWESNGQPENNYKTTPPVLDSDGSFFLYSKLTVDKSRWQQGNVFSCSVMHEALHNHYTQKSLSLS

SEQ ID NO: 3 - protein, 208 aa, synthetic construct
  source 1..208: note = Fc region of IgG2
GPSVFLFPPKPKDTLMISRTPEVTCVVVDVSHEDPEVQFNWYVDGVEVHNAKTKPREEQFNSTFRVVSVLTVVHQDWLNGKEYKCKVSNKGLPAPIEKTISKTKGQPREPQVYTLPPSREEMTKNQVSLTCLVKGFYPSDIAVEWESNGQPENNYKTTPPMLDSDGSFFLYSKLTVDKSRWQQGNVFSCSVMHEALHNHYTQKSLSLS

SEQ ID NO: 4 - protein, 208 aa, synthetic construct
  source 1..208: note = Fc region of IgG4
GPSVFLFPPKPKDTLMISRTPEVTCVVVDVSQEDPEVQFNWYVDGVEVHNAKTKPREEQFNSTYRVVSVLTVLHQDWLNGKEYKCKVSNKGLPSSIEKTISKAKGQPREPQVYTLPPSQEEMTKNQVSLTCLVKGFYPSDIAVEWESNGQPENNYKTTPPVLDSDGSFFLYSRLTVDKSRWQEGNVFSCSVMHEALHNHYTQKSLSLS

SEQ ID NO: 5 - protein, 208 aa, synthetic construct
  source 1..208: note = Fc region of IgG3
GPSVFLFPPKPKDTLMISRTPEVTCVVVDVSHEDPEVQFKWYVDGVEVHNAKTKPREEQYNSTFRVVSVLTVLHQDWLNGKEYKCKVSNKALPAPIEKTISKTKGQPREPQVYTLPPSREEMTKNQVSLTCLVKGFYPSDIAVEWESSGQPENNYNTTPPMLDSDGSFFLYSKLTVDKSRWQQGNIFSCSVMHEALHNHFTQKSLSLS

SEQ ID NO: 6 - protein, 7 aa, synthetic construct
  source 1..7: note = interaction site of Fc binding substance
KPKDTLM

SEQ ID NO: 7 - protein, 8 aa, synthetic construct
  source 1..8: note = interaction site of Fc binding substance
MHEALHNH

SEQ ID NO: 8 - protein, 9 aa, synthetic construct
  source 1..9: note = interaction site of Fc binding substance
MHEALHNHY

SEQ ID NO: 9 - protein, 16 aa, synthetic construct
  source 1..16: note = binding site of Fc binding substance
GPSVFLFPPKPKDTLM

SEQ ID NO: 10 - protein, 5 aa, synthetic construct
  source 1..5: note = CDRH1 of Claudin18.2 antibody
TYGVH

SEQ ID NO: 11 - protein, 16 aa, synthetic construct
  source 1..16: note = CDRH2 of Claudin18.2 antibody
VIWAGGSTNYNSALMS

SEQ ID NO: 12 - protein, 10 aa, synthetic construct
  source 1..10: note = CDRH3 of Claudin18.2 antibody
AAYYGNGLDY

SEQ ID NO: 13 - protein, 17 aa, synthetic construct
  source 1..17: note = CDRL1 of Claudin18.2 antibody
KSSQTLLNSGNQKNYLT

SEQ ID NO: 14 - protein, 7 aa, synthetic construct
  source 1..7: note = CDRL2 of Claudin18.2 antibody
WASTGES

SEQ ID NO: 15 - protein, 9 aa, synthetic construct
  source 1..9: note = CDRL3 of Claudin18.2 antibody
QNAYFYPFT

SEQ ID NO: 16 - protein, 448 aa, synthetic construct
  source 1..448: note = heavy chain of Claudin18.2 antibody
QVQLVESGGGVVQPGRSLRLSCAASGFSLTTYGVHWVRQAPGKGLEWVAVIWAGGSTNYNSALMSRFTISRDNSKNTLYLQMNSLRAEDTAVYYCARAAYYGNGLDYWGQGTMVTVSSASTKGPSVFPLAPSSKSTSGGTAALGCLVKDYFPEPVTVSWNSGALTSGVHTFPAVLQSSGLYSLSSVVTVPSSSLGTQTYICNVNHKPSNTKVDKRVEPKSCDKTHTCPPCPAPELLGGPSVFLFPPKPKDTLMISRTPEVTCVVVDVSHEDPEVKFNWYVDGVEVHNAKTKPREEQYNSTYRVVSVLTVLHQDWLNGKEYKCKVSNKALPAPIEKTISKAKGQPREPQVYTLPPSRDELTKNQVSLTCLVKGFYPSDIAVEWESNGQPENNYKTTPPVLDSDGSFFLYSKLTVDKSRWQQGNVFSCSVMHEALHNHYTQKSLSLSPGK

SEQ ID NO: 17 - protein, 220 aa, synthetic construct
  source 1..220: note = light chain of Claudin18.2 antibody
DIVMTQSPLSLPVTPGEPASISCKSSQTLLNSGNQKNYLTWYLQKPGQSPQLLIYWASTGESGVPDRFSGSGSGTDFTLKISRVEAEDVGVYYCQNAYFYPFTFGGGTKVEIKRTVAAPSVFIFPPSDEQLKSGTASVVCLLNNFYPREAKVQWKVDNALQSGNSQESVTEQDSKDSTYSLSSTLTLSKADYEKHKVYACEVTHQGLSSPVTKSFNRGEC

SEQ ID NO: 18 - DNA, 783 bp, synthetic construct
  source 1..783: mol_type = other DNA; note = nucleic acid encoding Claudin18.1 protein
atgtccaccaccacatgccaagtggtggcgttcctcctgtccatcctggggctggccggctgcatcgcggccaccgggatggacatgtggagcacccaggacctgtacgacaaccccgtcacctccgtgttccagtacgaagggctctggaggagctgcgtgaggcagagttcaggcttcaccgaatgcaggccctatttcaccatcctgggacttccagccatgctgcaggcagtgcgagccctgatgatcgtaggcatcgtcctgggtgccattggcctcctggtatccatctttgccctgaaatgcatccgcattggcagcatggaggactctgccaaagccaacatgacactgacctccgggatcatgttcattgtctcaggtctttgtgcaattgctggagtgtctgtgtttgccaacatgctggtgactaacttctggatgtccacagctaacatgtacaccggcatgggtgggatggtgcagactgttcagaccaggtacacatttggtgcggctctgttcgtgggctgggtcgctggaggcctcacactaattgggggtgtgatgatgtgcatcgcctgccggggcctggcaccagaagaaaccaactacaaagccgtttcttatcatgcctcaggccacagtgttgcctacaagcctggaggcttcaaggccagcactggctttgggtccaacaccaaaaacaagaagatatacgatggaggtgcccgcacagaggacgaggtacaatcttatccttccaagcacgactatgtg

SEQ ID NO: 19 - DNA, 786 bp, synthetic construct
  source 1..786: mol_type = other DNA; note = nucleic acid encoding Claudin18.2 protein
atggccgtgactgcctgtcagggcttggggttcgtggtttcactgattgggattgcgggcatcattgctgccacctgcatggaccagtggagcacccaagacttgtacaacaaccccgtaacagctgttttcaactaccaggggctgtggcgctcctgtgtccgagagagctctggcttcaccgagtgccggggctacttcaccctgctggggctgccagccatgctgcaggcagtgcgagccctgatgatcgtaggcatcgtcctgggtgccattggcctcctggtatccatctttgccctgaaatgcatccgcattggcagcatggaggactctgccaaagccaacatgacactgacctccgggatcatgttcattgtctcaggtctttgtgcaattgctggagtgtctgtgtttgccaacatgctggtgactaacttctggatgtccacagctaacatgtacaccggcatgggtgggatggtgcagactgttcagaccaggtacacatttggtgcggctctgttcgtgggctgggtcgctggaggcctcacactaattgggggtgtgatgatgtgcatcgcctgccggggcctggcaccagaagaaaccaactacaaagccgtttcttatcatgcctcaggccacagtgttgcctacaagcctggaggcttcaaggccagcactggctttgggtccaacaccaaaaacaagaagatatacgatggaggtgcccgcacagaggacgaggtacaatcttatccttccaagcacgactatgtgtaa